European Patent Specification EP 3 560 331 B1, published March 6, 2024. Title: Melon Plants with Melon Yellowing associated Virus (MYaV) Resistance. Applicant: Nunhems B.V. The sequence listing filed with the application follows.

SEQUENCE LISTING (30 sequences)

SEQ ID NO: 1 - DNA, 141 bp, Cucumis melo
  variation (71)..(71): SNP mME15090
cattatgatatctttctctcaactcaaccatgaactctaaagcaccattcccatctttcatctttcggtacgctcgcaaggctgtagagtaggatacgggagacagagttaggcctttcttcggcatctcttcaagaatgc

SEQ ID NO: 2 - DNA, 141 bp, Cucumis melo
  variation (71)..(71): SNP mME40332
ttgctgcaaagccaccaactccaggaattgttagcagaggaattgctttggagggtttctgtagtatcttggctggactctggggtacaggtgccggatcaactactttaacggaaaatgtacatactattcatgtaacaa

SEQ ID NO: 3 - DNA, 141 bp, Cucumis melo
  variation (71)..(71): mME12135
tgccagccgcacgtttcatcttttggtaataactattaaaagcataggaagcatgtgcttgaagggagttaggatcgtaacaagcgccaccctgttgaatggaacggcaatcagcctgtccttcaccacaagcatagtcca

SEQ ID NO: 4 - DNA, 141 bp, Cucumis melo
  variation (71)..(71): SNP mME28908
tccaatgtcatattttgatccgcagcatttgccttcatctggttgagtttagaataacaaacgtcagtattaaattacaacaaaccagckatattaccaaaaagaaaacaatcaatcagataaggaaaacctgaktggatt

SEQ ID NO: 5 - DNA, 139 bp, Cucumis melo
  variation (71)..(71): SNP mME36531
ctgttgaaatatattatgccgttattttcttggaatatttgctgtcaaatcctgtgttattgactggtcttttttgttaggtctacgctgaaggaccagctcgtcctactggtggggctgcatgtacgccgtctagact

SEQ ID NO: 6 - DNA, 141 bp, Cucumis melo
  variation (71)..(71): SNP mME9692
aagcacccctgtcattattttgcataatctcacaaagtcccccatcaacagaaccttcttcaacattgtcatcctcgcctatatcatcatctraaccagacacttccttctccaactgaggattgtaygtccattccaatc

SEQ ID NO: 7 - DNA, 141 bp, Cucumis melo
  variation (71)..(71): SNP mME50656
aaaaggggaagcaaaaagtttcgaaggaatcgcatgtttctgaagctcttgataagctcagagagcagaccagagaggcggttaaggggcttgaatcagtgtcaggtcctaaacctggtgttgatgaatttggtaaagatg

SEQ ID NO: 8 - DNA, 141 bp, Cucumis melo
  variation (71)..(71): SNP mME21377
tgtatcaggaacatagccagctgctttcatcttctctggcaacgcctccaagaacatgtagatttccttgacttgagggtgagatgtatcgccaccgagaaacatatgtgctttgccatttatctcgatccaactgcaacc

SEQ ID NO: 9 - DNA, 141 bp, Cucumis melo; identical to SEQ ID NO: 1
  variation (71)..(71): SNP mME15090

SEQ ID NO: 10 - DNA, 141 bp, Cucumis melo; identical to SEQ ID NO: 3
  variation (71)..(71): SNP mME12135

SEQ ID NO: 11 - DNA, 141 bp, Cucumis melo
  variation (71)..(71): SNP mME36533
ctataatacttcaataaataacatgcatacatacatacatggataatatagagagaagacaaggatagcttaagtttagtagttttgaagatgtgaatctcgatttttatctactacactgtttgaatggaatccttttct

SEQ ID NO: 12 - DNA, 141 bp, Cucumis melo
  variation (71)..(71): SNP mME13585
catattattcttaaataatataaaccacataattattaaattaaattgaactaaaactaccctattttaatgctttacaaactcttatctaatgtatgcttcatttaattatttttttggttgatactttcattttatttt

SEQ ID NO: 13 - DNA, 42 bp, Artificial Sequence
  mME12135 primer - allele FAM(dye)
gaaggtgaccaagttcatgctggtggcgcttgttacgatcct

SEQ ID NO: 14 - DNA, 42 bp, Artificial Sequence
  mME12135 pprimer -allele VIC(dye)
gaaggtcggagtcaacggattggtggcgcttgttacgatccc

SEQ ID NO: 15 - DNA, 25 bp, Artificial Sequence
  mME12135 Primer Common
aggaagcatgtgcttgaagggagtt

SEQ ID NO: 16 - DNA, 47 bp, artificial sequence
  mME36531
gaaggtgaccaagttcatgctcaaatcctgtgttattgactggtctc

SEQ ID NO: 17 - DNA, 47 bp, Artificial Sequence
  mME36531 Primer allele VIC(dye)
gaaggtcggagtcaacggattcaaatcctgtgttattgactggtctt

SEQ ID NO: 18 - DNA, 25 bp, Artificial Sequence
  mME36531 Primer Common
ggtccttcagcgtagacctaacaaa

SEQ ID NO: 19 - DNA, 44 bp, Artificial Sequence
  mME21377 Primer allele FAM(dye)
gaaggtgaccaagttcatgctggcgatacatctcaccctcaagt

SEQ ID NO: 20 - DNA, 43 bp, Artificial Sequence
  mME21377 Primer allele VIC(dye)
gaaggtcggagtcaacggattgcgatacatctcaccctcaagc

SEQ ID NO: 21 - DNA, 25 bp, Artificial Sequence
  mME21377 Primer Common
gcaacgcctccaagaacatgtagat

SEQ ID NO: 22 - DNA, 41 bp, Artificial Sequence
  mME15090 Primer allele FAM(dye)
gaaggtgaccaagttcatgctactctacagccttgcgagct

SEQ ID NO: 23 - DNA, 41 bp, Artificial Sequence
  mME15090 Primer allele VIC(dye)
gaaggtcggagtcaacggattactctacagccttgcgagcg

SEQ ID NO: 24 - DNA, 29 bp, Artificial Sequence
  mME15090 Primer Common
ctaaagcaccattcccatctttcatcttt

SEQ ID NO: 25 - DNA, 51 bp, Artificial Sequence
  mME36533 Primer alllel FAM(dye)
gaaggtgaccaagttcatgctagattcacatcttcaaaactactaaacttc

SEQ ID NO: 26 - DNA, 52 bp, Artificial Sequence
  mME36533 Primer allele VIC(dye)
gaaggtcggagtcaacggattgagattcacatcttcaaaactactaaactta

SEQ ID NO: 27 - DNA, 30 bp, Artificial Sequence
  mME36533 Primer Common
catggataatatagagagaagacaaggata

SEQ ID NO: 28 - DNA, 50 bp, Artificial Sequence
  mME13585 Primer allele FAM(dye)
gaaggtgaccaagttcatgctgcatacattagataagagtttgtaaagcg

SEQ ID NO: 29 - DNA, 51 bp, Artificial Sequence
  mME13585 Primer allele VIC(dye)
gaaggtcggagtcaacggattagcatacattagataagagtttgtaaagca

SEQ ID NO: 30 - DNA, 30 bp, Artificial Sequence
  mME13585 Primer Common
ttaaattgaactaaaactaccctattttaa